European Patent Application EP 4 692 365 A1, published February 11, 2026. Title: GENES, PROTEINS, AND PROCESSES FOR THE SYNTHESIS OF BLUE ANTHOCYANINS IN EUKARYOTIC CELLS. Applicant: Leibniz-Institut fuer Pflanzenbiochemie (IPB). The sequence listing filed with the application follows.

SEQUENCE LISTING (27 sequences)

SEQ ID NO: 1 - protein, 464 aa, Veronica persica
MPTTPTISVTIHEHCPIAPPAGDDQVSELNLPLSYFDVSWMNFPPASCLLFYRFPCSSVHFHETVVLNLKKSLSQTLKHYLPLAGNLLVPLSLDMPEFRYVKGDTLRFTIAEANVDFDFDYWTGNQARDAAQFHAFVPDLPEPKIDTDTGFRIMPVQSVQVTLLPGTGICFGFASDHAALDARSLVMFVKCWSSLTKLGKEDGELLAKNGLLPLFDRSVIIDPSNERANIFWDQMKQKPRFPKKLPVDVVRQTFVLQKSDLQKLRNSALAKRPGLVHLSSFTILSAYIWTCHVKAATKLGEEVNENEPEYYVIAMDGRHRLDPPVPAEYFGNCITPAVVASTHGQLKGEDGFCTAVELIGETISKLNSTEEFMKNNADDWLGKIKHVFRFQRNLTLAGSPKFDLYDTDFGWGTPNKYEVISIDGDNSLSLCKSREFEGGLELGLSLPKSKVDAFATFFVEGLKL

SEQ ID NO: 2 - protein, 452 aa, Veronica persica
MEKEEAKMFKILMFPWLAHGHIFPFLELAKTLSKRNFTIHFCSTAINLDSIKSNLANDPSVLDDSIKLLELEIESPELPPELHTTKNLPPHQFPLLIKDFENSKSSFFSIFDTLKPDMLIYDVFNPWAAKHALSHGSPSVWFMASGATICSFHYHQHLHKTGSLVPYEGVDFGEIKRHISPNTKGADFGGFILGSLNSSSEIILLKTSKELEKKYIDYLSFLCRKQIIPTGLLIANSDEKDEPEIMQWLDEKSERSTVYISFGSECFLSKEQIEEVAKGLELSNVNFIWIIRFPEGKNSMTVENALPEGFLERVKGRGMVIWKFAPQTRILAHKSIGGFVSHCGWSSITESVYFGVPIIAMPMKFEQVVNGVVVVEVGVGVEVEKDGSGQYLGEEVAKALDKVFGDNEFSKEVRYRASNLSDKIRENEEQEEDKVAEQLMSLCAKNKLQKCD

SEQ ID NO: 3 - protein, 466 aa, Veronica persica
MATTPAKRITIHKHCRVAPPVGDGEVVEQVLKTTYMDMPWVYFNPIQCVLFFRFPCSKVHFDETIIPNLKQSLSQALKHYLIVAGNVYIPLESGMPELRYVSGDSVSFIIAESDGDIEFDYLTGNHPRDACQFYEFVPYLPELKIDPDNEFKTMPVLSAQVTLFPDKGLSLGWATHHVAGDATSFIRFLKAWSSLANVGKDVDTYDFLAKNSLHSLFDRSVIADPSGRRANIYWNQIKKSGRIAPPPKLPTDKLRQTFGLTKSDMQKLRNSALAKKPWLVHLSTYTIVSAYLWSCFVKIASKIGEEVDAQEPEFFLMSVDARARLEPPVPLEYYGNCIVPAVVGSTHGELKGDDGFSNAVELIGDVISKQINNKEEFMKSADNQLERIRPIFGKRLLTVNGLPNFDMYGTDFGFGKTYKYEVLSIDGANCMSLCKSRDSEGGSEIGLTLPKPKLDAFASIFSEGLN

SEQ ID NO: 4 - protein, 465 aa, Veronica persica
MAGPRILVATFPAQGHINPSLQFAKRLIKMGSEVTFLISDYASHRIAGTTGGVYPKGLTVVSIPDGFGQKPADGDEKKHMEQMKSRGLKAVRDTLLEGVEQGRRFSCLVYSHLFAAAAEVARETKTPSALLWIEPATVLDIYYFYFNGYKDEIDKGDEIKLPGLPLLAQRDLPTFLLPSMPERFRLFMKEKLDILDAAEKPKVLINTFDVLEPDAINAIHKYEMVGIGPLIPSAYLDGLDPSDRSFGGDLVKKSEDSYLQWLSTNSESSVVYVSFGSGVMLPLPQLEEIAEALLKCGRPFLWVVRVNEDNERPEVEKLSCFKELEKLGKILTWCSQLEVLTHHSLGCFVTHCGWNSALESIALGVPVVAFPQFFDQGTNAKLIEDVWRTGVRVNRNEDKCVGRDEISRCIEMVMDGGERSQEMRENARKWKGLARESMEENGSSNKNLKAFLDELGDDEVIAVSQ

SEQ ID NO: 5 - protein, 464 aa, Veronica persica
MTISTNKVTVHAHCGVAPPVEMTEQRLSLTYFDMTWVHFHPIQRLIFYKFPCSTVQFYETIVPNLKESLSQTLKHFLPLAGNLYLPILNNPGFPEFRYVPGDTVSVTIAESSEDFDFDYWTGNHARDADEFYGFVPELSEPKIDSDSGLKIIPLVAVQVTVFPGTGISLGFTNNHAIGDANSIVRFIKSWATVSKLGKDADDAFLTKNELLPFFDRSVIKDPSQKRANIFWTEMKKRLSFVPPPSFPTNKFRETFILQQSDLQRLRIAAITKKPGLDYLSSFTISVAYVWSCIVKTASKSGEEVDENAAECILFSADARPRMDPPAPASYFGNCLVGVVTESTHGKLKGEEGFCTAVELIGELITKQVNNKDELLKDADEWLVKYKPLFGKRVFGVSGSPKFDLYDTDFGWGKAHKCESISIDKDSSLSICKSREFKGGLEIGMSLSKLKLDTFAAVFANGLEK

SEQ ID NO: 6 - DNA, 1395 bp, Veronica persica
  source 1..1395: mol_type = genomic DNA
atgccaacaacacctacaataagtgtcacaatacacgaacactgccctatcgcaccgcctgctggcgacgaccaagtgtcggagttaaaccttcctctgtcatacttcgacgtgtcatggatgaactttccgcccgcttcgtgtctccttttctaccggttcccctgttccagcgttcatttccatgaaaccgtagttcttaatctgaaaaaatcgttatctcaaactcttaaacactaccttcccctcgcaggcaacttattagttccgttgagtttagacatgcctgagtttcgctatgtcaagggagacactcttcgtttcacaattgcagaggcaaatgttgattttgatttcgactactggacaggaaatcaagctcgtgatgcagctcaattccacgctttcgtgcctgatttacccgaacccaagattgatactgacacaggtttcagaataatgcctgtccaatcagtacaagtgacgcttttgccaggaacagggatatgttttggatttgccagtgatcatgctgctctggatgctcgttcacttgttatgtttgtcaagtgttggagttcactaaccaagcttggaaaggaagatggtgaattactagccaaaaatggtttacttccactgtttgacagatcagtgatcatagatccatccaatgaacgagcaaatatattttgggatcaaatgaagcaaaagcctaggttcccgaaaaagttgcctgtggatgttgttaggcaaacatttgtgttacagaaaagtgatctacaaaaactcaggaactcagcgttagctaaacggccaggactagttcatttatcttctttcactattctgtcggcttacatttggacttgccatgtaaaagccgcaacaaaacttggtgaagaggtcaatgaaaacgaaccagaatactatgtcattgccatggatggtagacatcgtctggatccaccagttcctgcagaatatttcggcaattgcataactccagcagtggtagcatcaacacacggacagctgaaaggagaagatggtttttgcaccgcggttgagttaataggcgagactataagtaaacttaacagcacagaagagttcatgaaaaataatgctgatgactggctagggaagatcaagcatgtatttaggttccaaaggaacttaacactagctggatcaccgaaattcgacctgtatgatactgatttcgggtggggaacaccaaacaaatacgaagtgatttcgattgatggagataactctctgtctctctgtaaatcaagagagtttgaaggaggattggaacttggtttatctctgcctaagtctaaagtggacgctttcgctactttcttcgtggagggtctgaaactataa

SEQ ID NO: 7 - DNA, 1359 bp, Veronica persica
  source 1..1359: mol_type = genomic DNA
atggagaaagaagaagcaaaaatgttcaaaattctcatgtttccatggttagctcatggacacattttccctttccttgaacttgctaaaacactctccaaaagaaactttaccatacacttttgttccactgccattaatcttgattcaatcaagtccaaccttgctaatgatccatctgttcttgatgattcaataaagctactcgaactcgagatcgaatctcctgaactccctcctgaactccacacaactaagaacttaccaccacatcaatttcctctcttgataaaagactttgaaaactcaaaatcaagtttcttctccattttcgatactttaaagcccgatatgctgatttacgatgttttcaatccgtgggcagccaaacacgcgttatctcacggttcgccttctgtttggttcatggcatcaggtgctactatatgttcttttcattatcatcagcatttgcacaaaactggttcgcttgttccttatgagggagttgatttcggcgagatcaagcgtcacattagtccaaacactaaaggcgctgatttcggaggatttatattgggaagtttgaattcgtcttccgaaatcatcttgctaaagacctcaaaagaacttgaaaagaaatacattgattatctatcgtttttatgcaggaaacagattatacctactggtctactgattgcaaattctgatgagaaagatgagccagaaatcatgcaatggttagacgaaaaaagtgaacgttcgacggtctacatatcttttggtagcgagtgcttcttgtcgaaagaacagatcgaagaggtggccaaagggttggaactaagtaatgtgaattttatatggatcataagattccctgaaggaaagaatagtatgactgttgaaaacgcattgcctgaaggattcttagaaagggtgaaagggcgagggatggtgatttggaaattcgcgccacaaacgagaatattggcacataaaagtattggtggtttcgtgagtcactgcgggtggagttctataactgaaagcgtgtattttggagtaccgattatagccatgcctatgaaatttgagcaagtggtaaatggtgttgttgtggtggaggtgggcgttggagtagaggtcgaaaaggacgggagtggtcagtatttgggagaagaggtggcaaaagcattagataaggtgtttggggataatgagtttagtaaagaggtgagatacagagccagtaatttaagtgacaaaattcgcgagaatgaagaacaagaagaggataaagtagcagagcagctgatgagcctatgtgcgaagaacaagttgcagaaatgtgattga

SEQ ID NO: 8 - DNA, 1401 bp, Veronica persica
  source 1..1401: mol_type = genomic DNA
atggctactacacccgcaaagcgtataacaatacacaagcactgccgcgttgcaccaccagttggtgatggcgaagtggtagaacaagtccttaagacgacttacatggacatgccatgggtctactttaatcccatccaatgtgtactcttcttccggttcccctgttccaaagttcattttgacgaaaccataatcccgaatctcaaacaatctctctctcaagcactcaaacattaccttatcgtagctggcaatgtatacattcctttggaatccggcatgccggaattacgctatgtttctggcgactctgtttctttcataatagctgagtcagatggtgacattgaattcgactacttgacagggaaccatcctcgtgatgcctgtcaattctacgagtttgtgccttacttacctgaactaaaaatagatccagataatgagttcaagacaatgcccgtcttgtccgcccaggtgactctcttcccagacaaaggattaagtcttggctgggccacccatcacgttgctggagatgctacttcattcatcagatttctcaaggcctggagttcactagccaacgttgggaaagatgttgatacttatgacttcttagctaaaaattccttacattcacttttcgatagatccgtgattgcagatccatctgggcggcgagcaaatatttattggaaccaaataaaaaagtcgggcaggatagctcccccaccaaagttgcctactgataaacttaggcaaacatttggtctaacaaaaagtgacatgcaaaaactcaggaactcagcgttagctaaaaagccgtggttagtccacttgtcaacatatactatcgtttctgcatacctttggagttgctttgtgaaaattgcatcaaaaattggggaagaggtagatgcacaggagcctgaattctttctcatgtccgtggatgctcgggcacgtctggaaccacctgttccattagagtattacggaaattgcatagttccagcagtggtaggatcaactcacggagaattgaaaggagatgatggattttccaatgcggtcgagttaataggggatgttattagcaaacagataaataacaaggaggaattcatgaaaagtgctgataaccagctagagagaataaggcctatatttggcaaaaggcttttaacagtcaacggattgccaaacttcgacatgtatggtacagacttcgggtttggtaaaacatacaagtacgaagtgctttccatcgatggggcaaactgcatgtctctttgtaagtcaagagattccgagggagggtcagaaattggtttaactctgcctaaaccgaaactggatgcttttgcgtctatcttctccgaaggactaaactag

SEQ ID NO: 9 - DNA, 1398 bp, Veronica persica
  source 1..1398: mol_type = genomic DNA
atggcgggacctcgaatcttagtagcaacatttccagcacaaggccatatcaacccatccctccagttcgccaagagactcataaaaatgggaagtgaagtcacatttctcataagcgactatgcatcgcaccgcattgcaggaactactggcggtgtatatccaaagggactgacagtcgtgtcaattcctgatggttttggacaaaaaccggcagatggtgatgaaaagaaacatatggagcagatgaaaagtcgcgggttaaaggccgttcgggatactcttcttgagggggtagagcaaggccgacgattctcttgccttgtctactctcacctctttgctgcggcagctgaagtagcacgtgagactaaaaccccgagtgcgcttctctggattgaaccagccaccgtgttggatatatactatttctatttcaatgggtataaggatgaaattgacaagggtgatgaaattaagcttcctggtctgcctctattggcccaacgcgatcttccaacgtttctacttccttctatgcccgagaggtttcggttatttatgaaggagaagttggatatattggatgcggccgagaaacccaaggtgttgattaatacatttgatgtattggagcctgatgcaatcaatgccattcataagtacgagatggttggaatcggacccttgattccttccgcgtacttggacggtctagacccctcggatagatcattcgggggagatcttgttaaaaaatcagaggatagttacctccaatggctgagcactaactccgagtcgtcagtagtgtatgtgtctttcgggagcggggtgatgttgcctttgccacaactcgaggagatagcagaagcgctgttaaaatgtggcagaccgtttttgtgggtggtacgagtgaacgaggataatgaacgtccggaggttgagaaattgagctgtttcaaagagcttgaaaaacttggtaaaatattgacatggtgctcgcagttggaggttctaacacaccattcattgggatgttttgttactcactgcggttggaactctgcacttgagagcatagcgcttggtgtcccagttgtggcctttccacaattttttgatcaggggacgaatgccaagttaatagaagatgtgtggagaaccggagttcgtgtgaacaggaatgaagataaatgtgttggcagagacgagattagtagatgcattgagatggtgatggatggtggcgaaagaagccaagaaatgagagaaaatgcaaggaaatggaagggattggcaagggaatccatggaagaaaatggatcttcaaataagaacctaaaggcttttcttgatgagcttggagatgatgaagtcattgcagtttctcagtag

SEQ ID NO: 10 - DNA, 1395 bp, Veronica persica
  source 1..1395: mol_type = genomic DNA
atgactatctccacaaacaaagtaactgtccacgcgcactgtggcgttgcgccgccagtagagatgacagagcaacgcctttcgctgacatacttcgacatgacatgggtgcattttcatccaatccagcgtcttatcttctacaaattcccttgttccactgttcagttttatgaaaccatagtcccaaatctcaaagaatctctttctcaaactctcaaacacttccttcccttagcaggaaacttgtaccttccaatactaaacaatccaggatttcctgaatttcgatacgttcctggagacactgtttctgtcacgattgcagagtcaagtgaagattttgatttcgactactggactggaaaccacgctcgtgatgctgatgaattctatggctttgttcctgaattatctgaaccaaagatagattctgattccggcttaaaaataatcccactggtagccgttcaagtgacggtttttccaggaactgggatttctcttggatttaccaacaatcatgctattggggatgcgaattcgattgtgagattcattaagtcgtgggctacggtttccaagctcgggaaagatgccgatgatgcatttctaactaaaaatgagctacttccatttttcgacaggtcagtgatcaaagatccatctcaaaagcgtgcgaacatattttggactgaaatgaagaaacgcctaagttttgtcccacctcccagttttcctactaataaattcagggaaactttcattctccaacaaagtgatctgcagagactcagaatcgctgcgataaccaagaaaccggggttagactacttatcatcgtttactatttcagttgcttatgtttggagttgcatcgttaaaactgcatctaaaagtggagaagaggtcgatgaaaatgcggccgaatgcattctcttctcagcggatgcacgacctaggatggaccctccagcccctgcttcttactttggcaactgcttagttggggttgtgacagaatcaacacatggaaagctaaaaggagaagaaggattttgcaccgcggttgagttgataggcgagcttatcactaaacaggttaacaacaaggatgagttgttgaaagatgcagatgagtggctagtgaagtacaagcctttgtttggaaaacgagtatttggggtcagtggatcgccaaaattcgacctgtatgatacagactttggctggggaaaagcgcacaagtgcgagtcgatttccattgataaggatagttcattgtcaatttgtaagtcgagagaattcaagggaggattggagattggtatgtctttgtctaagctgaaactggacacttttgctgctgttttcgctaatgggttggagaagtaa

SEQ ID NO: 11 - DNA, 1427 bp, synthetic construct
  source 1..1427: mol_type = other DNA
atgctaacaagctctccattcatggtgttaaagtttcatttttcactgcatctggcaatgcaaacagagtgaaatctatgttgaactctgctccaactactagtatcgtccctctcactcttccgcaagtcgaaggtctacctcctggtgctgaaagtactgctgaattgacaccagtaactgctgaacttctcaaagttgctttagaccaaatgcaaccacaaatcaagtctttactttccaatctcagaccccattttgttcttttcgactttgctcaagattggctccctaaaatggctgatgaattggggatcaaatctgtttattactctgtttttgttgcactctccactgcttttcttacttgtcctgctagagtccctcaacccaaaaattgtccatctcttgaggacatgaaaaaacctccacctgcatttcctcacacctctgttacctcagtcaaaacctttgaagctcaagattttctatacattttcaagagtttccatggaggtcctacagaggtaaatccccagatgaacatggcatcgtggtgattgatgaaactgctgctgtcggctttaacctctctttaggcattggtttcgaagcgggcaacaagccgaaagaactgtacagcgaagaggcagtcaacggggaaactcagcaagcgcacttacaggcgattaaagagctgatagcgcgtgacaaaaaccacccaagcgtggtgatgtggagtattgccaacgaaccggatacccgtccgcaaggtgcacgggaatatttcgcgccactggcggaagcaacgcgtaaactcgacccgacgcgtccgatcacctgcgtcaatgtaatgttctgcgacgctcacaccgataccatcagcgatctctttgatgggcaggctgtaggacctccatggaaactcttgaaaatgtatagaaaatcttgagcttcaaaggttttgactgaggtaacagaggtgtgaggaaatgcaggtggaggttttttcatgtcctcaagagatggacaatttttgggttgagggactctagcaggacaagtaagaaaagcagtggagagtgcaacaaaaacagagtaataaacagatttgatccccaattcatcagccattttagggagccaatcttgagcaaagtcgaaaagaacaaaatggggtctgagattggaaagtaaagacttgatttgtggttgcatttggtctaaagcaactttgagaagttcagcagttactggtgtcaattcagcagtactttcagcaccaggaggtagaccttcgacttgcggaagagtgagagggacgatactagtagttggagcagagttcaacatagatttcactctgtttgcattgccagatgcagtgaaaaatgaaactttaacaccatgaatggagagcttgttag

SEQ ID NO: 12 - DNA, 23 bp, Lycopersicon esculentum
  source 1..23: mol_type = genomic DNA
caggagaattagaagaacgatgg

SEQ ID NO: 13 - DNA, 23 bp, Lycopersicon esculentum
  source 1..23: mol_type = genomic DNA
atgggtgtgcctcgagatgaagg

SEQ ID NO: 14 - DNA, 20 bp, synthetic construct
  source 1..20: mol_type = other DNA
caggagaattagaagaacga

SEQ ID NO: 15 - DNA, 20 bp, synthetic construct
  source 1..20: mol_type = other DNA
atgggtgtgcctcgagatga

SEQ ID NO: 16 - DNA, 47 bp, synthetic construct
  source 1..47: mol_type = other DNA
catttacaattatcgatacaatgccaacaacacctacaataagtgtc

SEQ ID NO: 17 - DNA, 47 bp, synthetic construct
  source 1..47: mol_type = other DNA
gcttgactctagaggatcaagcttatagtttcagaccctccacgaag

SEQ ID NO: 18 - DNA, 54 bp, synthetic construct
  source 1..54: mol_type = other DNA
catttacaattatcgatacaatggagaaagaagaagcaaaaatgttcaaaattc

SEQ ID NO: 19 - DNA, 51 bp, synthetic construct
  source 1..51: mol_type = other DNA
gcttgactctagaggatcaagctcagtcacattgttgcaacttgttcttcg

SEQ ID NO: 20 - DNA, 43 bp, synthetic construct
  source 1..43: mol_type = other DNA
catttacaattatcgatacaatggctactacacccgcaaagcg

SEQ ID NO: 21 - DNA, 51 bp, synthetic construct
  source 1..51: mol_type = other DNA
gcttgactctagaggatcaagctagtttagtccttcggagaagatagacgc

SEQ ID NO: 22 - DNA, 46 bp, synthetic construct
  source 1..46: mol_type = other DNA
catttacaattatcgatacaatggcgggacctcgaatcttagtagc

SEQ ID NO: 23 - DNA, 49 bp, synthetic construct
  source 1..49: mol_type = other DNA
gcttgactctagaggatcaagcctactgagaaactgcaatgacttcatc

SEQ ID NO: 24 - DNA, 51 bp, synthetic construct
  source 1..51: mol_type = other DNA
catttacaattatcgatacaatgactatctccacaaacaaagtaactgtcc

SEQ ID NO: 25 - DNA, 51 bp, synthetic construct
  source 1..51: mol_type = other DNA
gcttgactctagaggatcaagcttacttctccaacccattagcgaaaacag

SEQ ID NO: 26 - protein, 22 aa, synthetic construct
GSGATNFSLLKQAGDVEENPGP

SEQ ID NO: 27 - DNA, 22631 bp, synthetic construct
  source 1..22631: mol_type = other DNA
tgatgggctgcctgtatcgagtggtgattttgtgccgagctgccggtcggggagctgttggctggctggtggcaggatatattgtggtgtaaacaaattgacgcttagacaacttaataacacattgcggacgtttttaatgtactggggttgaacactctgtgaagacaatgccgaattcggatccggagagcggagaattaagggagtcacgttatgacccccgccgatgacgcgggacaagccgttttacgtttggaactgacagaaccgcaacgttgaaggagccactcagccgcgggtttctggagtttaatgagctaagcacatacgtcagaaaccattattgcgcgttcaaaagtcgcctaaggtcactatcagctagcaaatatttcttgtcaaaaatgctccactgacgttccataaattcccctcggtatccaattagagtctcatattcactctcaatccaaataatctgcaccggatctggatcgtttcgcatgattgaacaagatggattgcacgcaggttctccggccgcttgggtggagaggctattcggctatgactgggcacaacagacaatcggctgctctgatgccgccgtgttccggctgtcagcgcaggggcgcccggttctttttgtcaagaccgacctgtccggtgccctgaatgaactccaggacgaggcagcgcggctatcgtggctggccacgacgggcgttccttgcgcagctgtgctcgacgttgtcactgaagcgggaagggactggctgctattgggcgaagtgccggggcaggatctcctgtcatctcaccttgctcctgccgagaaagtatccatcatggctgatgcaatgcggcggctgcatacgcttgatccggctacctgcccattcgaccaccaagcgaaacatcgcatcgagcgagcacgtactcggatggaagccggtcttgtcgatcaggatgatctggacgaagagcatcaggggctcgcgccagccgaactgttcgccaggctcaaggcgcgtatgcccgacggcgaggatctcgtcgtgactcatggcgatgcctgcttgccgaatatcatggtggaaaatggccgcttttctggattcatcgactgtggccggctgggtgtggcggaccgctatcaggacatagcgttggctacccgtgatattgctgaagagcttggcggcgaatgggctgaccgcttcctcgtgctttacggtatcgccgctcccgattcgcagcgcatcgccttctatcgccttcttgacgagttcttctgagcgggactctggatctagagtcaagcagatcgttcaaacatttggcaataaagtttcttaagattgaatcctgttgccggtcttgcgatgattatcatataatttctgttgaattacgttaagcatgtaataattaacatgtaatgcatgacgttatttatgagatgggtttttatgattagagtcccgcaattatacatttaatacgcgatagaaaacaaaatatagcgcgcaaactaggataaattatcgcgcgcggtgtcatctatgttactagatcgacgctgcaagaattcaagcttggagttttgtggaagtgagagagtccaattttgataagaaaagagtcagaaaacgtaatattttaaaagtctaaatctttctacaaataagagcaaatttatttattttttaatccaataaatattaatggaggacaaattcaattcacttggttgtaaaataaacttaaaccaataaccaaagaactaataaatcctgaagtggaattattaaggataaatgtacatagacaatgaagaaataataggttcgatgaattaataataattaaggatgttacaatcatcatgtgccaagtatatacacaatattctatgggatttataatttcgttacttcacttaacttttgcgtaaataaaacgaattatctgatattttataataaaacagttaattaagaaccatcatttttaacaacatagatatattatttctaatagtttaatgatacttttaaatcttttaaattttatgtttctttagaaaataaaaattcaaaaaattaaatatatttacaaaaactacaatcaaacacaacttcatatattaaaagcaaaatatattttgaaaatttcaagtgtcctaacaaataagacaagaggaaaatgtacgatgagagacataaagagaactaataattgaggagtcctataatatataataaagtttattagtaaacttaattattaaggactcctaaaatatatgataggagaaaatgaatggtgagagatattggaaaacttaataattaaggattttaaaatatatggtaaaagataggcaaagtatccattatccccttttaacttgaagtctactaggcgcatgtgaaagttgattttttgtcacgtcatatagctataacgtaaaaaaagaaagtaaaatttttaattttttttaatatatgacatattttaaacgaaatataggacaaaatgtaaatgaatagtaaaggaaacaaagattaatacttactttgtaagaatttaagataaatttaaaatttaatagatcaactttacgtctagaaagacccatatctagaaggaatttcacgaaatcggcccttattcaaaaataacttttaaataatgaattttaaattttaagaaataatatccaatgaataaatgacatgtagcattttacctaaatatttcaactattttaatccaatattaatttgttttattcccaacaatagaaagtcttgtgcagacatttaatctgacttttccagtactaaatattaattttctgaagattttcgggtttagtccacaagttttagtgagaagttttgctcaaaattttaggtgagaaggtttgatatttatcttttgttaaattaatttatctaggtgactattatttatttaagtagaaattcatatcattacttttgccaacttgtagtcataataggagtaggtgtatatgatgaaggaataaacaagttcagtgaagtgattaaaataaaatataatttaggtgtacatcaaataaaaaccttaaagtttagaaaggcaccgaataattttgcatagaagatattagtaaatttataaaaataaaagaaatgtagttgtcaagttgtgttcttttttttggataaaaatagcagttggcttatgtcattcttttacaacctccatgccacttgtccaattgttgacacttaactaattagtttgattcatgtatgaatactaaataattttttaggactgactcaaatatttttatattatcatagtaatatttatctaatttttaggaccacttattactaaataataaattaactactactatattattgttgtgaaacaacaacgttttggttgttatgatgaaacgtacactatatcagtatgaaaaattcaaaacgattagtataaattatattgaaaatttgatatttttctattcttaatcagacgtattgggtttcatattttaaaaagggactaaacttagaagagaagtttgtttgaaactacttttgtctctttcttgttcccatttctctcttagatttcaaaaagtgaactactttatctctttctttgttcacattttattttattctattataaatatggcatcctcatattgagatttttagaaattattctaatcattcacagtgcaaaagaaaatggaaaagaattgtcgtggagtgagaaaaggtacttggaccaaagaagaggacactctcttgaggcaatgtatagaagagtatggtgaagggaaatggcatcaagttccacacagagcagggttgaaccggtgtaggaagagttgcaggctgaggtggttgaattatctgaggccaaatatcaaaagaggtcggttttcgagagatgaagtggacctaattgtgaggcttcataagctgttgggtaacaaatggtcgctgattgctggtagaattcctggaaggacagctaatgacgtgaagaacttttggaatactcatgtggggaagaatttaggcgaggatggagaacgatgccggaaaaatgttatgaacacaaaaaccattaagctgactaatatcgtaagaccccgagctcggaccttcaccggattgcacgttacttggccgagagaagtcggaaaaaccgatgaattttcaaatgtccggttaacaactgatgagattccagattgtgagaagcaaacgcaattttacaatgatgttgcgtcgccacaagatgaagttgaggactgcattcagtggtggagtaagttgctagaaacaacggaggatggggaattaggaaacctattcgaggaggcccaacaaattggaaattgagcttctctagctagagtcgatcgacaagctcgagtttctccataataatgtgtgagtagttcccagataagggaattagggttcctatagggtttcgctcatgtgttgagcatataagaaacccttagtatgtatttgtatttgtaaaatacttctatcaataaaatttctaattcctaaaaccaaaatccagtactaaaatccagatcgctactagaattcgagctcggagttttgtggaagtgagagagtccaattttgataagaaaagagtcagaaaacgtaatattttaaaagtctaaatctttctacaaataagagcaaatttatttattttttaatccaataaatattaatggaggacaaattcaattcacttggttgtaaaataaacttaaaccaataaccaaagaactaataaatcctgaagtggaattattaaggataaatgtacatagacaatgaagaaataataggttcgatgaattaataataattaaggatgttacaatcatcatgtgccaagtatatacacaatattctatgggatttataatttcgttacttcacttaacttttgcgtaaataaaacgaattatctgatattttataataaaacagttaattaagaaccatcatttttaacaacatagatatattatttctaatagtttaatgatacttttaaatcttttaaattttatgtttctttagaaaataaaaattcaaaaaattaaatatatttacaaaaactacaatcaaacacaacttcatatattaaaagcaaaatatattttgaaaatttcaagtgtcctaacaaataagacaagaggaaaatgtacgatgagagacataaagagaactaataattgaggagtcctataatatataataaagtttattagtaaacttaattattaaggactcctaaaatatatgataggagaaaatgaatggtgagagatattggaaaacttaataattaaggattttaaaatatatggtaaaagataggcaaagtatccattatccccttttaacttgaagtctactaggcgcatgtgaaagttgattttttgtcacgtcatatagctataacgtaaaaaaagaaagtaaaatttttaattttttttaatatatgacatattttaaacgaaatataggacaaaatgtaaatgaatagtaaaggaaacaaagattaatacttactttgtaagaatttaagataaatttaaaatttaatagatcaactttacgtctagaaagacccatatctagaaggaatttcacgaaatcggcccttattcaaaaataacttttaaataatgaattttaaattttaagaaataatatccaatgaataaatgacatgtagcattttacctaaatatttcaactattttaatccaatattaatttgttttattcccaacaatagaaagtcttgtgcagacatttaatctgacttttccagtactaaatattaattttctgaagattttcgggtttagtccacaagttttagtgagaagttttgctcaaaattttaggtgagaaggtttgatatttatcttttgttaaattaatttatctaggtgactattatttatttaagtagaaattcatatcattacttttgccaacttgtagtcataataggagtaggtgtatatgatgaaggaataaacaagttcagtgaagtgattaaaataaaatataatttaggtgtacatcaaataaaaaccttaaagtttagaaaggcaccgaataattttgcatagaagatattagtaaatttataaaaataaaagaaatgtagttgtcaagttgtgttcttttttttggataaaaatagcagttggcttatgtcattcttttacaacctccatgccacttgtccaattgttgacacttaactaattagtttgattcatgtatgaatactaaataattttttaggactgactcaaatatttttatattatcatagtaatatttatctaatttttaggaccacttattactaaataataaattaactactactatattattgttgtgaaacaacaacgttttggttgttatgatgaaacgtacactatatcagtatgaaaaattcaaaacgattagtataaattatattgaaaatttgatatttttctattcttaatcagacgtattgggtttcatattttaaaaagggactaaacttagaagagaagtttgtttgaaactacttttgtctctttcttgttcccatttctctcttagatttcaaaaagtgaactactttatctctttctttgttcacattttattttattctattataaatatggcatcctcatattgagatttttagaaattattctaatcattcacagtgcaaaagaaaatggctactggtatccaaaaccaaaagatagtgcctgagaatttgaggaagcaacttgctattgctgttagaagtatccaatggagttatgcaattttctggtccaattcagttgcacaaccaggggtcttggagtggggtgatgggttctacaatggagatattaaaactcgaaaaactgtacaatctgtcgaattgaatcccgatcagctgggattgcagagaagtgatcaattgagagaactttatgagtctctttcacttggtgaaaccaacacacaagctaaaaggcctactgctgcattatcaccagaggacctcactgatgctgagtggtttttcttggtttgcatgtctttcatattcaatattggccaagggttgcctggaagaacattagcacgaaatcaagcagtatggctatgcaacgctcatcgtgcggacaccaaagttttctcgcgttctttgcttgcaaagagtgcgtcaattcagacagttgtgtgctttccatatgcagaaggagtagttgagctgggagcaacagagctagtaccggaggatttgaatctaatccagcatataaaaacttcattcttggacagtcctgccaccgttcccaagattcccaactatgtctccaacagtattacaaacaacaatgacctcatttgtgaagcgcttgaacatgctaatataccagaaaacgatcttgatcagcttttgaattgtccagacacgaacatatgttctcctgataacagtttggatgactttgcagacaatttactcatagacgaatcgaatttggcagaaggcatcaatggggaggttcctcaaacacaaagctggcctttcatggatgatgcaatcagcaattgtctcaatagttctatgaattctagtgactgtatatctcaaactcatgaaaatctagagtcttttgccccactttctgatggaaaagggccaccggaaacgaataattgtatgcacagcactcaagaatgcaatcagcagatagaaaacacgggtgtccaaggcgatgaggtccattatcaaggggtactttccaatcttttgaagagttcccatcagttggttcttggtccctacttcagaaatgggaatagagaatcaagcttcgttagttggaacaaggatggatcgtcgggtactcatgttccccgaagcggaacctcacaaagatttctgaagaaagtactttttgaagtagctagaatgcatgaaaactccaggcttgatgctggtaaacaaaaaggcaacagtgactgccttgcaaagccaacggctgatgaaattgatagaaaccacgtcttgtcagagagaaaacgcagagagaaaataaacgaacggtttatgattcttgcatccctagtcccatccggtggcaaggttgacaaagtatcaatactagaccatacaatagattacttgagagggcttgagaggaaagtcgacgagctggaatctaacaaaatggtaaagggccgggggcgggaatcaactacaaaaactaaactgcacgatgccattgagaggacctccgataattatggcacaacaaggacaagtaatgtcaagaaaccgttgacaaacaagagaaaggcttctgatacggacaagattggagccgtaaatagcagaggtcgattgaaagattccttaacagataatataactgtgaacattacaaacaaggatgtgttgattgtcgtgagttgttcttccaaggagtttgtattgcttgaagtgatggaagccgtaagacgactaagtttggattccgaaactgttcaatcttccaacagagatggaattatatccattaccataaaagccaagtgcaagggattgaaggttgcatcagcaagtgtgatcaaacaagctcttcagaaagttactatgaagtcttgagcttaactttctgcacaaaaaaaaggatgaagatgactttataaatgtttgtgaaatctgttgaaatattcccttgttttgcttttgtgagatgtttttgtgtaaaatgtctttaaatggttcgttctacgattgcaataataattagtggtgctcattgttttggatggatcaatgttatacttatatcatttgaaaatctcatgattgttggacttggaccatagttgttaatttgaaggtttctaggttctaacgttaataatcttgttcaaaccaaataaatctcattacacaatttggggaggtgttaaaagattaccaaaataggttaattacaaattcgactatttccagtaatatgggctaatataggctccaatttagatactaataatgggctttataaagcccatttatttttctccttaatatcatcactcgcagagattacgcagcgggacgctttacaggggcaactccgtccagagaattcgcatgcggagtaaagcacgttaggtttagtagaagatttagacaaaatgattaacggatatgtgtttgattaagagtattgaaactttgtaatgattgttattcttgattgaagtagaaatctttgagaaccccaaaaacgtcacttagttttgtagtttttttctctgaatctttcttatttattatgcaagtcaaaagtggttgttgggaagagaagtgttcctctcatttacaacaaaaattcgatagcgatatatagtaatcgaaattttattcccaaacaagggaactttgttattgatagttggaactaaaagtttgtagagaaatttcaatgatacatatccaccgttagaggaacaaccaccacatgttctacccaaccctcacaacaaccagtttcttcaaatcttgagtctaataaaatgccaacacatctactctcatttcttctcatttataaaccagtttgatagacaagatattaataagtgcatatagtaaaatctttcttattcgtaacaaagttattgtaaacttatagaatgccaacaacacctacaataagtgtcacaatacacgaacactgccctatcgcaccgcctgctggcgacgaccaagtgtcggagttaaaccttcctctgtcatacttcgacgtgtcatggatgaactttccgcccgcttcgtgtctccttttctaccggttcccctgttccagcgttcatttccatgaaaccgtagttcttaatctgaaaaaatcgttatctcaaactcttaaacactaccttcccctcgcaggcaacttattagttccgttgagtttagacatgcctgagtttcgctatgtcaagggagacactcttcgtttcacaattgcagaggcaaatgttgattttgatttcgactactggacaggaaatcaagctcgtgatgcagctcaattccacgctttcgtgcctgatttacccgaacccaagattgatactgacacaggtttcagaataatgcctgtccaatcagtacaagtgacgcttttgccaggaacagggatatgttttggatttgccagtgatcatgctgctctggatgctcgttcacttgttatgtttgtcaagtgttggagttcactaaccaagcttggaaaggaagatggtgaattactagccaaaaatggtttacttccactgtttgacagatcagtgatcatagatccatccaatgaacgagcaaatatattttgggatcaaatgaagcaaaagcctaggttcccgaaaaagttgcctgtggatgttgttaggcaaacatttgtgttacagaaaagtgatctacaaaaactcaggaactcagcgttagctaaacggccaggactagttcatttatcttctttcactattctgtcggcttacatttggacttgccatgtaaaagccgcaacaaaacttggtgaagaggtcaatgaaaacgaaccagaatactatgtcattgccatggatggtagacatcgtctggatccaccagttcctgcagaatatttcggcaattgcataactccagcagtggtagcatcaacacacggacagctgaaaggagaagatggtttttgcaccgcggttgagttaataggcgagactataagtaaacttaacagcacagaagagttcatgaaaaataatgctgatgactggctagggaagatcaagcatgtatttaggttccaaaggaacttaacactagctggatcaccgaaattcgacctgtatgatactgatttcgggtggggaacaccaaacaaatacgaagtgatttcgattgatggagataactctctgtctctctgtaaatcaagagagtttgaaggaggattggaacttggtttatctctgcctaagtctaaagtggacgctttcgctactttcttcgtggagggtctgaaactataagcttggactcccatgttggcaaaggcaaccaaacaaacaatgaatgatccgctcctgcatatggggcggtttgagtatttcaactgccatttgggctgaattgtagacatgctcctgtcagaaattccgtgatcttactcaatattcagtaatctcggccaatatcctaaatgtgcgtggctttatctgtctttgtattgtttcatcaattcatgtaacgtttgcttttcttatgaattttcaaataaattatccgcttgtggaattcctcgagggagccgttggatccgttctctcatggaaaaagtagacgtctttgttctgtatgggcctttgactaactaaatggcccagcccgttcataacattaatcatttaaaaaatcacattgatggtataacactaattttttttttcacaggtgtataaccaactaatataaatatgcacattcacttaaaattaactaatatcataaagagtattatggcgtctgttttattgtttatccataactacatcaatcaaatccaagttgatatactagttagaacctaatactttacaaatccgatcattaatttatcttgtctgcttaagattttttttttgtgaataaggtttaattatctcatcaatacgatttagtaaaaagtctgtgcaaaaattaatgacgattgggatttttgtaacgcaagcccgtaccagaacatgtctccgccacgtgatttctccacagaccacaagcatttttaagacgtggctttctatcaaccgttaaaaacgtaaatcatattaaccatgtgtctactacctacggtgtaaacgaaactgtataacgtccctatcatataatagtaatgtgatacgttggaatgtagccaaaaagcataaaaaataaatagataattaagtttataatgttttcctacaaaatattattataccgtatgtattttttattttattttctgaagttaaaaacagatgtagttagttgagtaaattgtgttctagaaagagaagagagagcagtagtaccgtggtaggtagctagcgacctcttcgttcgtcagtcatcacaagctttgaaagattttcagctaccactctctcctttatatattcattacacatctcttctttctatatctctcttaatttagtcttttgtgttcgtaattacaatggctactacacccgcaaagcgtataacaatacacaagcactgccgcgttgcaccaccagttggtgatggcgaagtggtagaacaagtccttaagacgacttacatggacatgccatgggtctactttaatcccatccaatgtgtactcttcttccggttcccctgttccaaagttcattttgacgaaaccataatcccgaatctcaaacaatctctctctcaagcactcaaacattaccttatcgtagctggcaatgtatacattcctttggaatccggcatgccggaattacgctatgtttctggcgactctgtttctttcataatagctgagtcagatggtgacattgaattcgactacttgacagggaaccatcctcgtgatgcctgtcaattctacgagtttgtgccttacttacctgaactaaaaatagatccagataatgagttcaagacaatgcccgtcttgtccgcccaggtgactctcttcccagacaaaggattaagtcttggctgggccacccatcacgttgctggagatgctacttcattcatcagatttctcaaggcctggagttcactagccaacgttgggaaagatgttgatacttatgacttcttagctaaaaattccttacattcacttttcgatagatccgtgattgcagatccatctgggcggcgagcaaatatttattggaaccaaataaaaaagtcgggcaggatagctcccccaccaaagttgcctactgataaacttaggcaaacatttggtctaacaaaaagtgacatgcaaaaactcaggaactcagcgttagctaaaaagccgtggttagtccacttgtcaacatatactatcgtttctgcatacctttggagttgctttgtgaaaattgcatcaaaaattggggaagaggtagatgcacaggagcctgaattctttctcatgtccgtggatgctcgggcacgtctggaaccacctgttccattagagtattacggaaattgcatagttccagcagtggtaggatcaactcacggagaattgaaaggagatgatggattttccaatgcggtcgagttaataggggatgttattagcaaacagataaataacaaggaggaattcatgaaaagtgctgataaccagctagagagaataaggcctatatttggcaaaaggcttttaacagtcaacggattgccaaacttcgacatgtatggtacagacttcgggtttggtaaaacatacaagtacgaagtgctttccatcgatggggcaaactgcatgtctctttgtaagtcaagagattccgagggagggtcagaaattggtttaactctgcctaaaccgaaactggatgcttttgcgtctatcttctccgaaggactaaactagcttagagctttcgttcgtatcatcggtttcgacaacgttcgtcaagttcaatgcatcagtttcattgcgcacacaccagaatcctactgagtttgagtattatggcattgggaaaactgtttttcttgtaccatttgttgtgcttgtaatttactgtgttttttattcggttttcgctatcgaactgtgaaatggaaatggatggagaagagttaatgaatgatatggtccttttgttcattctcaaattaatattatttgttttttctcttatttgttgtgtgttgaatttgaaattataagagatatgcaaacattttgttttgagtaaaaatgtgtcaaatcgtggcctctaatgaccgaagttaatatgaggagtaaaacacttgtagttgtaccattatgcttattcactaggcaacaaatatattttcagacctagaaaagctgcaaatgttactgaatacaagtatgtcctcttgtgttttagacatttatgaactttcctttatgtaattttccagaatccttgtcagattctaatcattgctttataattatagttatactcatggatttgtagttgagtatgaaaatattttttaatgcattttatgacttgccaattgattgacaacgctgagcgaattccatatgggagcgagagttaccactttgacaatcgttcgtaaacaacctttgaattaagacataaaacgttgactgtgggattattaagcgtaacgaacaaataacgacttttaaatagagtctattaatttgcttaaaaagggggccgaatatttcaggcccatcaattaccacgtgaagtctggttttgcttttgttgatgttacgataccatcacgtgtttgcacttaccaggaggttacacttgcccggtcatttggttacccaataaccacacaccattcatcaggacactcaccaatctgatccgttaaaggtttatgtatttatacacatccaacacacaacttagaaattaacaaaagagaacaaaaaaagtctaataaggatcttccggtagttaaagtgaaatacaagagagtccaagaaaatggagaaagaagaagcaaaaatgttcaaaattctcatgtttccatggttagctcatggacacattttccctttccttgaacttgctaaaacactctccaaaagaaactttaccatacacttttgttccactgccattaatcttgattcaatcaagtccaaccttgctaatgatccatctgttcttgatgattcaataaagctactcgaactcgagatcgaatctcctgaactccctcctgaactccacacaactaagaacttaccaccacatcaatttcctctcttgataaaagactttgaaaactcaaaatcaagtttcttctccattttcgatactttaaagcccgatatgctgatttacgatgttttcaatccgtgggcagccaaacacgcgttatctcacggttcgccttctgtttggttcatggcatcaggtgctactatatgttcttttcattatcatcagcatttgcacaaaactggttcgcttgttccttatgagggagttgatttcggcgagatcaagcgtcacattagtccaaacactaaaggcgctgatttcggaggatttatattgggaagtttgaattcgtcgtccgaaatcatcttgctaaagacctcaaaagaacttgaaaagaaatacattgattatctatcgtttttatgcaggaaacagattatacctactggtctactgattgcaaattctgatgagaaagatgagccagaaatcatgcaatggttagacgaaaaaagtgaacgttcgacggtctacatatcttttggtagcgagtgcttcttgtcgaaagaacagatcgaagaggtggccaaagggttggaactaagtaatgtgaattttatatggatcataagattccctgaaggaaagaatagtatgactgttgaaaacgcattgcctgaaggattcttagaaagggtgaaagggcgagggatggtgatttggaaattcgcgccacaaacgagaatattggcacataaaagtattggtggtttcgtgagtcactgcgggtggagttctataactgaaagcgtgtattttggagtaccgattatagccatgcctatgaaatttgagcaagtggtaaatggtgttgttgtggtggaggtgggcgttggagtagaggtcgaaaaggacgggagtggtcagtatttgggagaagaggtggcaaaagcattagataaggtgtttggggataatgagtttagtaaagaggtgagatacagagccagtaatttaagtgacaaaattcgcgagaatgaagaacaagaagaggataaagtagcagagcagctgatgagcctatgtgcgaagaacaagttgcagaaatgtgattgagcttgtcctgctttaatgagatatgcgagaagcctatgatcgcatgatatttgctttcaattctgttgtgcacgttgtaaaaaacctgagcatgtgtagctcagatccttaccgccggtttcggttcattctaatgaatatatcacccgttactatcgtatttttatgaataatattctccgttcaatttactgattgtaccctactacttatatgtacaatattaaaatgaaaacaatatattgtgctgaataggtttatagcgacatctatgatagagcgccacaataacaaacaattgcgttttattattacaaatccaattttaaaaaaagcggcagaaccggtcaaacctaaaagactgattacataaatcttattcaaatttcaaaagtgccccaggggctagtatctacgacacaccgagcggcgaactaataacgctcactgaagggaactccggttccccgccggcgcgcatgggtgagattccttgaagttgagtattggccgtccgctctaccgaaagttacgggcaccattcaacccggtccagcacggcggccgggtaaccgacttgctgccccgagaattatgcagcatttttttggtgtatgtgggccccaaatgaagtgcaggtcaaaccttgacagtgacgacaaatcgttgggcgggtccagggcgaattttgcgacaacatgtcgaggctcagcaggaccgcttgccgaattcggatccggagctcgtggctgttactcgtcggtcgtcacataagacttttctcatccaccggtcttgtaagagacagacagtgcaaagattgtcaattattcctaatccatcttttataccattgatacttaaaatggtttagctcttatatataaaagcttgagtatgttctttcttttactaaaacttataacatcttcaaaacattctaaaatggcgggacctcgaatcttagtagcaacatttccagcacaaggccatatcaacccatccctccagttcgccaagagactcataaaaatgggaagtgaagtcacatttctcataagcgactatgcatcgcaccgcattgcaggaactactggcggtgtatatccaaagggactgacagtcgtgtcaattcctgatggttttggacaaaaaccggcagatggtgatgaaaagaaacatatggagcagatgaaaagtcgcgggttaaaggccgttcgggatactcttcttgagggggtagagcaaggccgacgattctcttgccttgtctactctcacctctttgctgcggcagctgaagtagcacgtgagactaaaaccccgagtgcgcttctctggattgaaccagccaccgtgttggatatatactatttctatttcaatgggtataaggatgaaattgacaagggtgatgaaattaagcttcctggtctgcctctattggcccaacgcgatcttccaacgtttctacttccttctatgcccgagaggtttcggttatttatgaaggagaagttggatatattggatgcggccgagaaacccaaggtgttgattaatacatttgatgtattggagcctgatgcaatcaatgccattcataagtacgagatggttggaatcggacccttgattccttccgcgtacttggacggtctagacccctcggatagatcattcgggggagatcttgttaaaaaatcagaggatagttacctccaatggctgagcactaactccgagtcgtcagtagtgtatgtgtctttcgggagcggggtgatgttgcctttgccacaactcgaggagatagcagaagcgctgttaaaatgtggcagaccgtttttgtgggtggtacgagtgaacgaggataatgaacgtccggaggttgagaaattgagctgtttcaaagagcttgaaaaacttggtaaaatattgacatggtgctcgcagttggaggttctaacacaccattcattgggatgttttgttactcactgcggttggaactctgcacttgagagcatagcgcttggtgtcccagttgtggcctttccacaattttttgatcaggggacgaatgccaagttaatagaagatgtgtggagaaccggagttcgtgtgaacaggaatgaagataaatgtgttggcagagacgagattagtagatgcattgagatggtgatggatggtggcgaaagaagccaagaaatgagagaaaatgcaaggaaatggaagggattggcaagggaatccatggaagaaaatggatcttcaaataagaacctaaaggcttttcttgatgagcttggagatgatgaagtcattgcagtttctcagtaggcttggaatgttaagaattgggttcaatgaccactggttaacggaggcctcaacaacttcgccaccaagcaaaaataaactaatgcaaacttacccaatatttaagtcacatccaagtgttggtgttgtatggccactaatcttggcagatatattgctgcagttctatcaataaaatttgaattttcgttgtgcaactctattcgctcatactttacattaagtctacctaaatgctttcactgaaattgttttggctttggtttataatgcagtcagccatgcggcccatgcctcattctcaattacgcccaaatccctagtcatcaattaattacttggccaaacaaacaagtcaaactatgtaatgatactcgattacaccccaattcagtttctgggaattaaaaatagatatggcttcaatttgcttgcaaaagagagaagaacatgagaacacaaatttacagcaattacaattcgaaacatattctttactcaatttatctatgctggttagaatcttacgttggttaacgctgcaagaattcaagcttggagccaactaagaccacatttatcatggtaatcatattatcaccactttttatcattcataataaatgttttacctattttctacatggttttgtgaagaactaaatccacattaacctgataacaatgttctcaccattattatcgataatcaaaacgttagcttccctcattttcacgatgtgtttggacgattaatatttctacatattgtaagtgtaactatattatctaggtaagcacacagttatcttgataaacatattatccccacttttaccgtttacccttaccgttacccatccacattaatatatacttaaactcttctcgtttcactttactgttgagggtttcatgaaaacataagacaccaattatcgtaataacagttttgtcaccattgtaatcgataatgcaaatgttagcaaatattctcattataaatgtttatgctgacagatcacataaattgtcttattatattatccaactaagactattgttatcatggtaaaacatattatcactacttttaccgttaactataaatgtcatctatccgtataatcatatatcttacattcttttccttttactctactctggaggatttcgtgatgatctaaaaaattaattgtgataacaatgttcttaccataatcaaggataataaaaatgttagcaaccaccctcataatttatgttccttgttatcattatctatatatgaaaatttattagactagtgatattcttatgtagataaatgtttttaaccaaagctagtttatgtttcttttatcaggtcacttaataaaaccacttttattctaacgatgactaatatgttcatgtagatcttatttggtcataggggcaatttcgtcttattattttctggtgacaaaaaacaactaaatatctgatttctatggatagatacttaattatttagttttctatgtatatatatttaactcacccttattaatttgtggttttttttgtttgggttttaaatgagctgcattataatttcaaaaaattagcccaacaatatgagagtagagtgttactgttgatttatatcgtaagatatttatttctaatgatatcaacaaaatttctgtaaacttaaaaataaaaattaaaacaaattcgtaaactgtttaatagttaccagaaaatataaattacatgaacttgaactagaaattcgcctccttttttagtccataaccttgtttataaatttggaaaagaaaaaactcaaacataaagcttatttaaaataaaataaaaaatagcatatataaatatacacccaccggttgggtaaacctagcaggtggttgatattcttgggagagaagtaagtaaggacccataacctccaaaagaagctaatatctatcctatagaagtatacatagtctaacgctcaaagccaaagtcaaaacaataaaactttgaaattcagtaatgactatctccacaaacaaagtaactgtccacgcgcactgtggcgttgcgccgccagtagagatgacagagcaacgcctttcgctgacatacttcgacatgacatgggtgcattttcatccaatccagcgtcttatcttctacaaattcccttgttccactgttcagttttatgaaaccatagtcccaaatctcaaagaatctctttctcaaactctcaaacacttccttcccttagcaggaaacttgtaccttccaatactaaacaatccaggatttcctgaatttcgatacgttcctggagacactgtttctgtcacgattgcagagtcaagtgaagattttgatttcgactactggactggaaaccacgctcgtgatgctgatgaattctatggctttgttcctgaattatctgaaccaaagatagattctgattccggcttaaaaataatcccactggtagccgttcaagtgacggtttttccaggaactgggatttctcttggatttaccaacaatcatgctattggggatgcgaattcgattgtgagattcattaagtcgtgggctacggtttccaagctcgggaaagatgccgatgatgcatttctaactaaaaatgagctacttccatttttcgacaggtcagtgatcaaagatccatctcaaaagcgtgcgaacatattttggactgaaatgaagaaacgcctaagttttgtcccacctcccagttttcctactaataaattcagggaaactttcattctccaacaaagtgatctgcagagactcagaatcgctgcgataaccaagaaaccggggttagactacttatcatcgtttactatttcagttgcttatgtttggagttgcatcgttaaaactgcatctaaaagtggagaagaggtcgatgaaaatgcggccgaatgcattctcttctcagcggatgcacgacctaggatggaccctccagcccctgcttcttactttggcaactgcttagttggggttgtgacagaatcaacacatggaaagctaaaaggagaagaaggattttgcaccgcggttgagttgataggcgagcttatcactaaacaggttaacaacaaggatgagttgttgaaagatgcagatgagtggctagtgaagtacaagcctttgtttggaaaacgagtatttggggtcagtggatcgccaaaattcgacctgtatgatacagactttggctggggaaaagcgcacaagtgcgagtcgatttccattgataaggatagttcattgtcaatttgtaagtcgagagaattcaagggaggattggagattggtatgtctttgtctaagctgaaactggacacttttgctgctgttttcgctaatgggttggagaagtaagcttattagctccaatttatgatgatctgaagaaccaaataagctttatagtttctgttttatgtttgtgttgttttgtacgtttcagtaataaattcaatatacttttaagattcatgtcaatgctaagaccatagttctctattcttaagtttttactctatttttgagtgagatataaaatggggttaaaatagaagtggagtttttacatagtatacaaggttactcacttgtactattattcgaatataagaagaacttctttctgtatgtatatcacaagattatttcatcaaccaaaaattgtatatcccctcattaggccaagagaactataactaaaataaaattaaaaaaaaaaatacttttttacattcagaaagataatgtaacattataagaatttgcttccccgctactattgtcttcgaggatgcacatgtgaccgagggacacgaagtgatccgtttaaactatcagtgtttgacaggatatattggcgggtaaacctaagagaaaagagcgtttattagaataatcggatatttaaaagggcgtgaaaaggtttatccgttcgtccatttgtatgtgcatgccaaccacagggttcccctcgggagt